European Patent Specification EP 4 408 978 B1, published April 15, 2026. Title: Stabilising the human spindle by KIFC1/HSET. Applicant: Max-Planck-Gesellschaft zur Forderung der Wissenschaften e.V. The sequence listing filed with the application follows.

SEQUENCE LISTING (94 sequences)

SEQ ID NO: 1 - protein, 673 aa, Homo sapiens
MDPQRSPLLEVKGNIELKRPLIKAPSQLPLSGSRLKRRPDQMEDGLEPEKKRTRGLGATTKITTSHPRVPSLTTVPQTQGQTTAQKVSKKTGPRCSTAIATGLKNQKPVPAVPVQKSGTSGVPPMAGGKKPSKRPAWDLKGQLCDLNAELKRCRERTQTLDQENQQLQDQLRDAQQQVKALGTERTTLEGHLAKVQAQAEQGQQELKNLRACVLELEERLSTQEGLVQELQKKQVELQEERRGLMSQLEEKERRLQTSEAALSSSQAEVASLRQETVAQAALLTEREERLHGLEMERRRLHNQLQELKGNIRVFCRVRPVLPGEPTPPPGLLLFPSGPGGPSDPPTRLSLSRSDERRGTLSGAPAPPTRHDFSFDRVFPPGSGQDEVFEEIAMLVQSALDGYPVCIFAYGQTGSGKTFTMEGGPGGDPQLEGLIPRALRHLFSVAQELSGQGWTYSFVASYVEIYNETVRDLLATGTRKGQGGECEIRRAGPGSEELTVTNARYVPVSCEKEVDALLHLARQNRAVARTAQNERSSRSHSVFQLQISGEHSSRGLQCGAPLSLVDLAGSERLDPGLALGPGERERLRETQAINSSLSTLGLVIMALSNKESHVPYRNSKLTYLLQNSLGGSAKMLMFVNISPLEENVSESLNSLRFASKVNQCVIGTAQANRK

SEQ ID NO: 2 - DNA, 2022 bp, Homo sapiens
  source 1..2022: mol_type = other DNA
atggatccgcagaggtcccccctattggaagtaaaggggaacatagaactgaagagacctctgattaaggccccttcccagctgcctctctcaggaagcagactcaagaggaggcctgaccagatggaagatggcctggagcctgagaagaaacggacaagaggcctgggtgcaacgaccaaaattaccacatcccacccaagagttccatccctcactacagtgccacagacacaaggccagaccacagctcaaaaagtttccaagaagacaggaccccggtgttccacagctattgccacagggttgaagaaccagaagccagttcctgctgttcctgtccagaagtctggcacatcaggtgttcctcccatggcaggagggaagaaacccagcaaacgtccagcctgggacttaaagggtcagttatgtgacctaaatgcagaactaaaacggtgccgtgagaggactcaaacgttggaccaagagaaccagcagcttcaggaccagctcagagatgcccagcagcaggtcaaggccctggggacagagcgcacaacactggaggggcatttagccaaggtacaggcccaggctgagcagggccaacaggagctgaagaacttgcgtgcttgtgtcctggagctggaagagcggctgagcacgcaggagggcttggtgcaagagcttcagaaaaaacaggtggaattgcaggaagaacggaggggactgatgtcccaactagaggagaaggagaggaggctgcagacatcagaagcagccctgtcaagcagccaagcagaggtggcatctctgcggcaggagactgtggcccaggcagccttactgactgagcgggaagaacgtcttcatgggctagaaatggagcgccggcgactgcacaaccagctgcaggaactcaagggcaacatccgtgtattctgccgggtccgccctgtcctgccgggggagcccactccaccccctggcctcctcctgtttccctctggccctggtgggccctctgatcctccaacccgccttagcctctcccggtctgacgagcggcgtgggaccctgagtggggcaccagctcccccaactcgccatgatttttcctttgaccgggtattcccaccaggaagtggacaggatgaagtgtttgaagagattgccatgcttgtccagtcagccctggatggctatccagtatgcatctttgcctatggccagacaggcagtggcaagaccttcacaatggagggtgggcctgggggagacccccagttggaggggctgatccctcgggccctgcggcacctcttctctgtggctcaggagctgagtggtcagggctggacctacagctttgtagcaagctacgtagagatctacaatgagactgtccgggacctgctggccactggaacccggaagggtcaagggggcgagtgtgagattcgccgtgcagggccagggagtgaggagctcactgtcaccaatgctcgatatgtccctgtctcctgtgagaaagaagtggacgccctgcttcatctggcccgccagaatcgggctgtggcccgcacagcccagaatgaacggtcatcacgcagccacagtgtattccagctacagatttctggggagcactccagccgaggcctgcagtgtggggcccccctcagtcttgtggacctggccgggagtgagcgacttgaccccggcttagccctcggccccggggagcgggaacgccttcgggaaacacaggccattaacagcagcctgtccacgctggggctggttatcatggccctgagcaacaaggagtcccacgtgccttaccggaacagcaaactgacctacctgctgcagaactctctgggtggtagtgctaagatgctcatgtttgtgaacatttctccactggaagagaacgtctccgagtccctcaactctctacgctttgcctccaaggtgaaccagtgtgttattggtactgctcaggccaacaggaagtga

SEQ ID NO: 3 - protein, 670 aa, Bos taurus
MEPQRSPLLEVKGNVELKRPLAKAASRLPLSGRRLKRGPDQMEEALEPEKKRTRGLGTRVTTTHPRAAALSSAPQTQGQTAVPKAPRKPAPRCSTAVAPVLKTQKPGPVVPVQKPGTTAAPPMVGGKKPKRPAWDLKGQLCDLNAELKCYRERKQVLDQENQQLRDQLQEAQQQALALGAERKTLEEELTRVRAQAEQGQRELGNLSARVLELEERLGTQEGLVQELQKEQLRLQEERRGLAARLGEQERRLQTSEASLSDSQEEVASLRQEAAAREAILAEREDRLHGLEMERRRLHNQLQELKGNIRVFCRVRPVLPGESTPSPGFLQFPSGPCGPSDPPTRLSLSRSDERRGTLSGAPAGPTRHEFSFDRVFPPGSGQDEVFEEISMLVQSALDGYPVCIFAYGQTGSGKTFTMEGGPGGDPQMEGLIPRALRHLFSVAQELSGQGWTYSFVASYVEIYNETVRDLLATGTRKGQGGECEIRRAGPGSEELTVTNARYVPVSCEREVEALLHLARQNRAVARTAQNERSSRSHSVFQLQISGEHASRGLQCAAPLSLVDLAGSERLDPGLALGPGERERLRETQAINSSLSTLGLVIMALSNKESHVPYRNSKLTYLLQNSLGGSAKMLMFVNISPLEENVSESLNSLRFASKVNQCVIGTAQANKK

SEQ ID NO: 4 - protein, 668 aa, Sus scrofa
METLQRSPLLEVKGNIEVKRPLPKPPSRLPLSGSRLKRGPEQMEEALEPEKKRTRGLGTKIAPSRPRAALLTAVPQTQGQAAARTAPKKTGPRCPTAVATVLKNQKPGPAVPAQKPGTAAPPMVGGKKPSKRPAWDLKGQLCDRMAELKCCRERNQILDQENQQLRDQLREAQQQASTLGAERRTLEEELARVRVQAEQGQQELGRLSAQVLELEERLGTQEGLVQVLQREQLGLQEERRGLATRLEEQERRLQASEAALSDSQAEVASLRQEAAAQAVLLAEREDRLHGLEMERRRLHNQLQELKGNIRVFCRVRPVLPGEPTPNPGFLLFPGGPADPPTRLSLSRSDERRGTLSGAPAPPTRHDFSFDRVFPPGSRQDEVFEEIAMLVQSALDGYPVCIFAYGQTGSGKTFTMEGGPAGDPQVEGLIPRALRHLFSVAQELSGQGWTYSFVASYVEIYNETVRDLLATGTRKGQAGECEIRRAGPGSEELTVTNARYVPVSCEKEVQALLHLARQNRAVARTAQNERSSRSHSVFQLQISGEHAARGLQCIAPLSLVDLAGSERLDSGLALGPGERERLRETQSINSSLSTLGLVIMALSNKEPHVPYRNSKLTYLLQNSLGGSAKMLMFVNISPLEENVSESLNSLRFASKVNQCVIGTAQANKK

SEQ ID NO: 5 - protein, 674 aa, Mus musculus
MDVQAQRPPLLEVKRNVELKAALVKSSSRVPLSASRLKRGPDQMEDALEPAKKRTRVMGAVTKVDTSRPRGPLLSTVSQTQGHTAAQKGPKKTGPRGCSAIGTVLRSQKPVPAAPAQKPGTSTAPVVVGKRAGKRPAWDLKGQLCDLNEELKRYREKTQTLELENRGLREQLREVQEQATTLGTERNTLEGELASVRSRAEQDQQRLETLSARVLELEECLGTRERLLQELQGERLQLQEERSTLSTQLEEQERRFQATEAALSSSQEEVVCLRQKTEAQVTLLAEQGDRLYGLEMERRRLHNQLQELKGNIRVFCRVRPVLEGESTPSPGFLVFPPGPAGPSDPPTGLSLSRSDDRRSTLTGAPAPTVRHDFSFDRVFPPGSKQEEVFEEIAMLVQSALDGYPVCIFAYGQTGSGKTFTMEGGPRGDPQLEGLIPRAMRHLFSVAQEMSGQGWTYSFVASYVEIYNETVRDLLATGPRKGQGGECEIRRASPGSEELTVTNARYVPVSCEKEVEALLHLAHQNRAVAHTAQNKRSSRSHSVFQLQISGEHAARGLQCGAPLNLVDLAGSERLDPGLHLGPGERDRLRETQAINSSLSTLGLVIMALSNKESHVPYRNSKLTYLLQNSLGGSAKMLMFVNISPLEENVSESLNSLRFASKVNQCVIGTAQANKK

SEQ ID NO: 6 - DNA, 2013 bp, Bos taurus
  source 1..2013: mol_type = other DNA
atggagccgcagaggtccccgttgttggaagtgaaggggaacgtagagctgaagagacccctggctaaggctgcttcccggctgcctctctcgggacgcaggctgaagagggggcctgaccagatggaggaggccttggagccggagaagaaaagaacacgaggcctgggcaccagagtgaccacgacccaccccagagcagcagccctcagctccgcgccacagacacaaggccagaccgcagtgcccaaagctcccaggaagccagcaccccgatgttccacggctgttgccccagtgctgaagactcagaagccaggtcctgttgttcccgtccagaagcctggaacgacagccgcacctcccatggtgggagggaagaaacccaaacgtccggcctgggacttaaaggggcagttatgtgacctcaatgcagagctgaaatgctaccgtgagaggaagcaggtgctggaccaggagaaccaacagctgcgggaccagctccaggaggcccagcaacaggccttggccctgggggcagagcgtaagaccctggaagaggagttgaccagggtgcgggcccaggctgagcagggccagcgggagctggggaacctgagtgcccgtgtcctggagctggaagagcggctgggcacgcaggagggcttagtgcaagagctccagaaggaacagctgagattgcaggaggagcgcaggggactggctgcccggctgggagagcaggagcggaggctgcagacctcagaagcttctctgtcggacagccaggaagaggtggcatctctgcgccaggaggctgcagcccgggaggccatactggctgagcgggaagaccgtctccacgggctcgagatggagcgcaggcggttacacaaccagctgcaggaactcaaaggcaacatccgtgtgttctgccgggtccgccccgtccttccaggggagtccaccccatcccctggcttcctccagtttccctctggcccctgtggaccctctgaccctccaacccgcctcagcctctcgcggtctgacgagcggcgtgggaccctgagtggggcgccagctggccctacccgccatgagttctcctttgaccgggtgttcccaccagggagtggacaggatgaagtgtttgaggagatttccatgcttgtccagtcagccctggatggctatccagtgtgcatctttgcttatggccagacaggcagtggcaagaccttcaccatggagggtgggcctgggggagacccccagatggaggggctgatccctcgtgccctgcgacacctcttttctgtggcccaggagctaagtggccagggctggacctacagctttgtggcaagttacgtagagatctacaacgagactgtccgagacctgctggccactgggacccggaagggccaggggggtgagtgtgagattcgccgggcagggccaggcagcgaggagctcactgtcaccaacgcgcgctatgttccggtctcctgtgagagggaggtggaagccctgctccatctagcccgccagaaccgcgctgtagcccgcacagcccagaatgagcgctcgtcgcgtagtcacagcgtgttccagctgcagatctctggggagcacgctagccgaggcctgcagtgtgcggcccccctcagcctggtggacttggctgggagtgagcggctagaccccggcttagcactcggccctggggagcgggaacgccttcgggaaacacaggccattaacagcagcctgtccacgctggggctggtcatcatggccttgagcaacaaggagtcccatgtgccttaccggaacagcaagctcacctacctgctgcagaactctctgggtggcagtgccaagatgctcatgtttgtgaacatttctcccctagaagagaacgtctccgagtccctcaactccctacgcttcgcctccaaggtgaaccagtgtgttattggcactgcccaggccaacaagaaatga

SEQ ID NO: 7 - DNA, 2007 bp, Sus scrofa
  source 1..2007: mol_type = other DNA
atggagacgctgcagaggtcgcccttgttggaagtgaaggggaacatagaggtaaagagacccctgcccaagcccccttcccggctgcccttgtcaggaagcagacttaagagggggcctgagcagatggaggaggccttggaacctgagaagaaaaggacgcgaggcctgggcaccaaaatcgccccgtcccgccccagagcagcgttgctcaccgcagtgcctcagacgcagggccaggctgcagcgcgcacggctcccaagaagacaggaccccgctgtcccacagctgttgccacagtgctgaagaatcagaagccaggccctgctgttcctgcccagaagcctggcacagctgcccctcccatggtgggagggaagaagcccagcaaacgtccggcctgggacttaaagggtcagttatgtgaccgaatggcagagctgaaatgctgccgtgagaggaatcagattttggatcaggagaaccaacagctgcgggaccagcttagggaggcccagcagcaggcctcgaccctgggcgcagagcgccggacactggaagaggagttggcccgggttcgggtccaggctgagcagggccagcaggagctggggaggctgagtgcccaggttctggagctggaggagcggctgggcacgcaggagggcttggtgcaagtgcttcagagagagcagctggggctgcaggaggagcggagggggctggccacccggctggaggagcaggagcggaggctgcaggcatcggaggcagcgctgtcggacagccaggcggaggtggcatctcttcgccaggaggctgcggcccaggcagtcttgctggccgagcgggaagaccgcctgcacgggctggagatggagcgccggcggctccacaaccagcttcaggagctcaaaggcaacatccgcgtgttctgccgtgtccgcccagtcctccctggggagcccaccccgaaccccggcttcctcctgttccctggcgggcccgctgaccctccaacacgcctcagcctctcccggtctgacgaacggcgtgggaccctgagtggggcaccggccccccccacgcgacacgacttctcctttgaccgggtcttcccaccagggagcaggcaggatgaagtgtttgaggagattgccatgcttgtgcagtctgccctggatggttacccagtgtgcatctttgcctatggccagaccggcagtggcaagaccttcaccatggagggtgggcctgcgggagacccccaggtggagggactgatcccccgggccctgcggcacctcttctctgtggcacaggagctcagtggccagggctggacctacagctttgtggccagttacgtcgagatctacaacgagactgtccgagacctgctggccactggaacccggaagggccaggcgggtgagtgtgagattcgccgggcagggccagggagtgaggagcttactgtcaccaacgcccgctacgttcctgtctcctgtgagaaagaggtacaggccctgctccatctggcccgccagaaccgggctgtggcccgcacagcccagaatgaacggtcatcacgcagtcatagcgtgttccagctgcagatctctggggaacacgcggcccgaggcctgcagtgcatcgccccgctcagtcttgtggacctggccgggagcgagcggctggattccggcctcgcccttggccctggggagcgggaacgccttcgggaaacacagtccattaacagcagcttgtccacactggggctggtcatcatggccttgagcaacaaggagccccatgtgccttaccggaacagcaagctcacctacctgctgcagaactctctgggtggcagcgctaagatgctcatgttcgtgaacatctcccccctggaagagaatgtctctgagtctctcaactccttgcgctttgcttccaaggtgaaccaatgtgtcattggtactgcccaagccaacaagaaatga

SEQ ID NO: 8 - DNA, 2025 bp, Mus musculus
  source 1..2025: mol_type = other DNA
atggacgtgcaggcgcagaggccacctttgttggaagtgaagaggaacgtagaactgaaggcagccctggtgaagtcctcctcccgagtgcccctgtcagcaagcaggctcaagaggggtcctgaccagatggaggatgccttggagcctgcaaagaaacggacacgagtcatgggtgcagtgaccaaagttgacacatcccgtcccagaggaccactcctcagcacagtgtcacagacccagggccacactgcagctcagaaaggccctaagaagacaggacctcgtgggtgctctgctattggtacagtgctgaggagccagaagccagttcccgctgctcctgcccagaagcctggcacatccactgctcctgtggtggtagggaagagagctggcaaacgccctgcctgggacctgaagggccagttgtgtgacctcaatgaagagttgaaacgctatcgggagaagactcaaacgctggaactggagaaccggggtcttcgggagcaactcagagaggtccaggagcaggccacgaccctggggacagagcggaacaccctggaaggggagctggccagtgtacgcagccgagctgagcaggaccagcagaggctggagacgctgagtgcccgtgtcttggagctggaggaatgtctgggtaccagggaaaggctgcttcaggagcttcagggagagcggctgcaattgcaggaggagcggagcacactgagcacccagctggaggagcaggagaggaggtttcaggccacagaagcagctctgtcaagcagccaagaagaggtggtgtgtcttcggcagaagactgaagcccaggtgaccttactggctgagcaaggagaccggctctatgggttagagatggagcggcgacgactccacaaccagctgcaggaactgaagggcaatatccgggtgttctgccgcgtgcgccctgtcctcgaaggggaatccactccatctcctggcttcctcgtgtttcctcctggccctgctggaccctctgatcccccgacgggccttagcctctcacgatctgatgatcggcgctccaccctgactggggccccggcccccactgtccgccatgatttctcctttgatcgggtgttcccgccgggaagcaagcaggaggaagtgtttgaggagatcgccatgcttgtccagtcagcactggatggctaccctgtgtgcatttttgcctatggacagacaggcagtggcaagaccttcactatggaaggagggcctaggggagacccccaattggaagggctgatccctcgggccatgcggcatctgttctctgtggcccaggagatgagcggccagggctggacatacagttttgtggcgagttacgtagagatctacaatgagaccgttcgagacctgctagctactgggccccgcaagggacaagggggcgagtgtgagatccgtcgggcaagcccaggaagtgaggagcttactgtcaccaatgcccgctatgtccctgtttcctgtgagaaagaggtggaggccctgctccatttggctcatcagaaccgggctgtggcccacactgcccaaaataagagatcatcacgcagtcatagtgtgttccagctgcagatttctggagagcatgcagctcggggcctgcagtgtggcgctccgctcaaccttgtggacctagctgggagtgagcggctagaccctggcttacacctaggccctggggagcgtgatcgtcttcgggagacacaggccattaacagcagtctgtctacactgggactggtcataatggccctgagcaataaggagtcccacgtgccttaccgaaacagcaagctcacctacttgctgcagaactctctgggtggcagtgccaagatgcttatgtttgtgaatatttctcctctggaagagaatgtctccgagtctctgaattcactacgctttgcttccaaggtgaaccagtgtgtcattggtactgctcaggctaataagaagtga

SEQ ID NO: 9 - protein, 673 aa, Macaca mulatta
MDPQRSPLLEVKGNIELKRPRIKAPSRLPLSGSRLKRRPDQMEDGLEPEKKRTRGLGATTKITTSHPRVPSLTTVPQTQGQTTAQKVSKKTGPRCSTAIATGLKNQKPVPAVPVQKPGTSAVPPMAGGKKPSKRPAWDLKGQLCDLNAELKRCRERTQTLDQENQQLQDQLRDAQQQAKALGTERRTLEGHLAKVQAQAEQGQQELKNLRACVLELEERLSTQEGLVQELQKKQVELQEERRGLTSQLEEKERRLQTSEAALSSSRAEVASLWQETAAQAALLAEREERLHGLEMERRRLHNQLQELKGNIRVFCRVRPVLPGEPTPPPGLLLFPSGPGGPSDPPTRLSLSRSDERRGTLSGAPAPPTRHDFSFDRVFPPGSGQDEVFEEIAMLVQSALDGYPVCIFAYGQTGSGKTFTMEGGPGGDPQLEGLIPRALRHLFSVAQELSGQGGTYSFVASYVEIYNETVRDLLATGTRKGQGGECEIRRAGPGSEELTVTNARYVPVSCEKEVEALLHLARQNRAVARTAQNERSSRSHSVFQLQISGEHSSRGLQCGASLSLVDLAGSERLDPGLALGPGERERLRETQAINSSLSTLGLVIMALSNKESHVPYRNSKLTYLLQNSLGGSAKMLMFVNISPLEENVSESLNSLRFASKVNQCVIGTAQANRK

SEQ ID NO: 10 - DNA, 21 bp, synthetic construct
  misc_feature 1..21: note = synthetic sequence
  source 1..21: mol_type = other DNA
aaggttgaaatcgaaattgaa

SEQ ID NO: 11 - DNA, 21 bp, synthetic construct
  misc_feature 1..21: note = synthetic sequence
  source 1..21: mol_type = other DNA
ttggaatttcttattagtaaa

SEQ ID NO: 12 - DNA, 21 bp, synthetic construct
  misc_feature 1..21: note = synthetic sequence
  source 1..21: mol_type = other DNA
caggagggttctagcatctta

SEQ ID NO: 13 - DNA, 21 bp, synthetic construct
  misc_feature 1..21: note = synthetic sequence
  source 1..21: mol_type = other DNA
cacaagaaatatctaacttta

SEQ ID NO: 14 - DNA, 21 bp, synthetic construct
  misc_feature 1..21: note = synthetic sequence
  source 1..21: mol_type = other DNA
caaggctacaatggtactata

SEQ ID NO: 15 - DNA, 21 bp, synthetic construct
  misc_feature 1..21: note = synthetic sequence
  source 1..21: mol_type = other DNA
aagcattgggctcgtgaataa

SEQ ID NO: 16 - DNA, 21 bp, synthetic construct
  misc_feature 1..21: note = synthetic sequence
  source 1..21: mol_type = other DNA
cagcaacttcttagtacacaa

SEQ ID NO: 17 - DNA, 21 bp, synthetic construct
  misc_feature 1..21: note = syntehtic sequence
  source 1..21: mol_type = other DNA
accgagagcagtgtacggaaa

SEQ ID NO: 18 - DNA, 21 bp, synthetic construct
  misc_feature 1..21: note = synthetic sequence
  source 1..21: mol_type = other DNA
caggttcgagacgcagcaata

SEQ ID NO: 19 - DNA, 21 bp, synthetic construct
  misc_feature 1..21: note = syntehtic sequence
  source 1..21: mol_type = other DNA
ctggtattgaatgtaacggaa

SEQ ID NO: 20 - DNA, 21 bp, synthetic construct
  misc_feature 1..21: note = synthetic sequence
  source 1..21: mol_type = other DNA
aaggaggatggtgacacaata

SEQ ID NO: 21 - DNA, 21 bp, synthetic construct
  misc_feature 1..21: note = synthetic sequence
  source 1..21: mol_type = other DNA
caggaagagttctaaccacaa

SEQ ID NO: 22 - DNA, 21 bp, synthetic construct
  misc_feature 1..21: note = synthetic sequence
  source 1..21: mol_type = other DNA
aacgccaagcttgaaggtaaa

SEQ ID NO: 23 - DNA, 21 bp, synthetic construct
  misc_feature 1..21: note = synthetic sequence
  source 1..21: mol_type = other DNA
aagatggatattgccaatcta

SEQ ID NO: 24 - DNA, 21 bp, synthetic construct
  misc_feature 1..21: note = synthetic sequence
  source 1..21: mol_type = other DNA
ccggatggagattatcaatga

SEQ ID NO: 25 - DNA, 21 bp, synthetic construct
  misc_feature 1..21: note = synthetic sequence
  source 1..21: mol_type = other DNA
ctggagaaattcaaagaccta

SEQ ID NO: 26 - DNA, 21 bp, synthetic construct
  misc_feature 1..21: note = synthetic sequence
  source 1..21: mol_type = other DNA
agcaaggattggagtcgctaa

SEQ ID NO: 27 - DNA, 21 bp, synthetic construct
  misc_feature 1..21: note = synthetic sequence
  source 1..21: mol_type = other DNA
cccgaacagtgtcatccacta

SEQ ID NO: 28 - DNA, 21 bp, synthetic construct
  misc_feature 1..21: note = synthetic sequence
  source 1..21: mol_type = other DNA
ctggacggattacaagatcaa

SEQ ID NO: 29 - DNA, 21 bp, synthetic construct
  source 1..21: mol_type = other DNA
atggattgtttctctgttgaa

SEQ ID NO: 30 - DNA, 21 bp, synthetic construct
  source 1..21: mol_type = other DNA
ttgagtggtattggtatatta

SEQ ID NO: 31 - DNA, 21 bp, synthetic construct
  misc_feature 1..21: note = synthetic sequence
  source 1..21: mol_type = other DNA
cagagtgatgttgatgggata

SEQ ID NO: 32 - DNA, 21 bp, synthetic construct
  misc_feature 1..21: note = synthetic sequence
  source 1..21: mol_type = other DNA
ccagaattagattctaattta

SEQ ID NO: 33 - DNA, 21 bp, synthetic construct
  misc_feature 1..21: note = synthetic sequence
  source 1..21: mol_type = other DNA
tagactgagaatttaattcta

SEQ ID NO: 34 - DNA, 21 bp, synthetic construct
  misc_feature 1..21: note = synthetic sequence
  source 1..21: mol_type = other DNA
aaggagtgcatccgagcctta

SEQ ID NO: 35 - DNA, 21 bp, synthetic construct
  misc_feature 1..21: note = synthetic sequence
  source 1..21: mol_type = other DNA
ctgctggaccattccatctta

SEQ ID NO: 36 - DNA, 21 bp, synthetic construct
  misc_feature 1..21: note = synthetic sequence
  source 1..21: mol_type = other DNA
caggatgttgatgctacaaat

SEQ ID NO: 37 - DNA, 21 bp, synthetic construct
  misc_feature 1..21: note = synthetic sequence
  source 1..21: mol_type = other DNA
caggaatggcatcctgtgaaa

SEQ ID NO: 38 - DNA, 21 bp, synthetic construct
  misc_feature 1..21: note = synthetic sequence
  source 1..21: mol_type = other DNA
aagaattggcttggaaatgaa

SEQ ID NO: 39 - DNA, 21 bp, synthetic construct
  misc_feature 1..21: note = synthetic sequence
  source 1..21: mol_type = other DNA
tacgatgaaatacatggtcaa

SEQ ID NO: 40 - DNA, 21 bp, synthetic construct
  misc_feature 1..21: note = synthetic sequence
  source 1..21: mol_type = other DNA
caggaactggagggtcaaata

SEQ ID NO: 41 - DNA, 21 bp, synthetic construct
  misc_feature 1..21: note = synthetic sequence
  source 1..21: mol_type = other DNA
agcaaagaacataatgaataa

SEQ ID NO: 42 - DNA, 21 bp, synthetic construct
  misc_feature 1..21: note = synthetic sequence
  source 1..21: mol_type = other DNA
cacaggaactttgccagttaa

SEQ ID NO: 43 - DNA, 21 bp, synthetic construct
  misc_feature 1..21: note = synthetic sequence
  source 1..21: mol_type = other DNA
ttccatcttgaacataaataa

SEQ ID NO: 44 - DNA, 21 bp, synthetic construct
  misc_feature 1..21: note = synthetic sequence
  source 1..21: mol_type = other DNA
aaggcatattagaaagggaaa

SEQ ID NO: 45 - DNA, 21 bp, synthetic construct
  misc_feature 1..21: note = synthetic sequence
  source 1..21: mol_type = other DNA
aaggcctctcttcttgttaaa

SEQ ID NO: 46 - DNA, 21 bp, synthetic construct
  misc_feature 1..21: note = synthetic sequence
  source 1..21: mol_type = other DNA
aacctgagtctcggttcacaa

SEQ ID NO: 47 - DNA, 21 bp, synthetic construct
  misc_feature 1..21: note = synthetic sequence
  source 1..21: mol_type = other DNA
ctggctggaactgggaaataa

SEQ ID NO: 48 - DNA, 21 bp, synthetic construct
  misc_feature 1..21: note = synthetic sequence
  source 1..21: mol_type = other DNA
atggattaagtttatgtgaaa

SEQ ID NO: 49 - DNA, 21 bp, synthetic construct
  misc_feature 1..21: note = synthetic sequence
  source 1..21: mol_type = other DNA
tcggcttgaggcagaaattaa

SEQ ID NO: 50 - DNA, 21 bp, synthetic construct
  misc_feature 1..21: note = synthetic sequence
  source 1..21: mol_type = other DNA
aagcagcatcttgaacaggaa

SEQ ID NO: 51 - DNA, 21 bp, synthetic construct
  misc_feature 1..21: note = synthetic sequence
  source 1..21: mol_type = other DNA
aggctggataatgatatatta

SEQ ID NO: 52 - DNA, 21 bp, synthetic construct
  misc_feature 1..21: note = synthetic sequence
  source 1..21: mol_type = other DNA
caggattcctacgataactta

SEQ ID NO: 53 - DNA, 21 bp, synthetic construct
  misc_feature 1..21: note = synthetic sequence
  source 1..21: mol_type = other DNA
cacaatagaatcaatggagaa

SEQ ID NO: 54 - DNA, 21 bp, synthetic construct
  misc_feature 1..21: note = synthetic sequence
  source 1..21: mol_type = other DNA
cacatggtagaactaaactaa

SEQ ID NO: 55 - DNA, 21 bp, synthetic construct
  misc_feature 1..21: note = synthetic sequence
  source 1..21: mol_type = other DNA
tgcattgtaaatattgtttaa

SEQ ID NO: 56 - DNA, 21 bp, synthetic construct
  misc_feature 1..21: note = synthetic sequence
  source 1..21: mol_type = other DNA
cagatttatttgcgacaacaa

SEQ ID NO: 57 - DNA, 21 bp, synthetic construct
  misc_feature 1..21: note = synthetic sequence
  source 1..21: mol_type = other DNA
ttggaggaaactgtcaaacta

SEQ ID NO: 58 - DNA, 21 bp, synthetic construct
  misc_feature 1..21: note = synthetic sequence
  source 1..21: mol_type = other DNA
caggaagttaaagctgaacta

SEQ ID NO: 59 - DNA, 21 bp, synthetic construct
  misc_feature 1..21: note = synthetic sequence
  source 1..21: mol_type = other DNA
cagctagatgaaacaagtcaa

SEQ ID NO: 60 - DNA, 21 bp, synthetic construct
  misc_feature 1..21: note = synthetic sequence
  source 1..21: mol_type = other DNA
ctcctttgccttgaagagtaa

SEQ ID NO: 61 - DNA, 21 bp, synthetic construct
  misc_feature 1..21: note = synthetic sequence
  source 1..21: mol_type = other DNA
aacggcaatccttacgtgaaa

SEQ ID NO: 62 - DNA, 21 bp, synthetic construct
  misc_feature 1..21: note = synthetic sequence
  source 1..21: mol_type = other DNA
aaggaggaaagtgctaacaaa

SEQ ID NO: 63 - DNA, 21 bp, synthetic construct
  misc_feature 1..21: note = synthetic sequence
  source 1..21: mol_type = other DNA
caggacttagatatgaaacaa

SEQ ID NO: 64 - DNA, 21 bp, synthetic construct
  misc_feature 1..21: note = synthetic sequence
  source 1..21: mol_type = other DNA
acggtagaagtaagtaaagaa

SEQ ID NO: 65 - DNA, 21 bp, synthetic construct
  misc_feature 1..21: note = synthetic sequence
  source 1..21: mol_type = other DNA
cagatagaagattctgaaata

SEQ ID NO: 66 - DNA, 21 bp, synthetic construct
  misc_feature 1..21: note = synthetic sequence
  source 1..21: mol_type = other DNA
aaggctgaagactatgaagaa

SEQ ID NO: 67 - DNA, 21 bp, synthetic construct
  misc_feature 1..21: note = synthetic sequence
  source 1..21: mol_type = other DNA
ttgtttgaatatgatctttaa

SEQ ID NO: 68 - DNA, 21 bp, synthetic construct
  misc_feature 1..21: note = synthetic sequence
  source 1..21: mol_type = other DNA
tacgatctatgaggaagataa

SEQ ID NO: 69 - DNA, 21 bp, synthetic construct
  misc_feature 1..21: note = synthetic sequence
  source 1..21: mol_type = other DNA
ctgagtcatcttgcagaagaa

SEQ ID NO: 70 - DNA, 21 bp, synthetic construct
  misc_feature 1..21: note = synthetic sequence
  source 1..21: mol_type = other DNA
tacactgggactggtcataat

SEQ ID NO: 71 - DNA, 21 bp, synthetic construct
  misc_feature 1..21: note = synthetic sequence
  source 1..21: mol_type = other DNA
gtgaacaatatttattatgta

SEQ ID NO: 72 - DNA, 21 bp, synthetic construct
  misc_feature 1..21: note = synthetic sequence
  source 1..21: mol_type = other DNA
cagagcctgattcccttgcaa

SEQ ID NO: 73 - DNA, 21 bp, synthetic construct
  misc_feature 1..21: note = synthetic sequence
  source 1..21: mol_type = other DNA
ctgcgcggaggttgaaattca

SEQ ID NO: 74 - DNA, 21 bp, synthetic construct
  misc_feature 1..21: note = synthetic sequence
  source 1..21: mol_type = other DNA
caggcatttgagagagggcaa

SEQ ID NO: 75 - DNA, 21 bp, synthetic construct
  misc_feature 1..21: note = synthetic sequence
  source 1..21: mol_type = other DNA
cagtgtctgcatcttcactta

SEQ ID NO: 76 - DNA, 21 bp, synthetic construct
  misc_feature 1..21: note = synthetic sequence
  source 1..21: mol_type = other DNA
cagtatggtggagatctacaa

SEQ ID NO: 77 - DNA, 21 bp, synthetic construct
  misc_feature 1..21: note = synthetic sequence
  source 1..21: mol_type = other DNA
ccgcaccaccgagttcaccaa

SEQ ID NO: 78 - DNA, 21 bp, synthetic construct
  misc_feature 1..21: note = synthetic sequence
  source 1..21: mol_type = other DNA
cagaggtctgggctatattta

SEQ ID NO: 79 - DNA, 21 bp, synthetic construct
  misc_feature 1..21: note = synthetic sequence
  source 1..21: mol_type = other DNA
gggcatgtatataatgttcta

SEQ ID NO: 80 - DNA, 21 bp, synthetic construct
  misc_feature 1..21: note = synthetic sequence
  source 1..21: mol_type = other DNA
caggataagaaatgtcttgaa

SEQ ID NO: 81 - DNA, 21 bp, synthetic construct
  misc_feature 1..21: note = synthetic sequence
  source 1..21: mol_type = other DNA
cagctggacactctaaagcaa

SEQ ID NO: 82 - DNA, 21 bp, synthetic construct
  misc_feature 1..21: note = synthetic sequence
  source 1..21: mol_type = other DNA
aatgttattacttgtaaataa

SEQ ID NO: 83 - DNA, 21 bp, synthetic construct
  misc_feature 1..21: note = synthetic sequence
  source 1..21: mol_type = other DNA
ctggaagtagaactagatcaa

SEQ ID NO: 84 - DNA, 21 bp, synthetic construct
  misc_feature 1..21: note = synthetic sequence
  source 1..21: mol_type = other DNA
aaggagatccatgcaaagcaa

SEQ ID NO: 85 - DNA, 21 bp, synthetic construct
  misc_feature 1..21: note = synthetic sequence
  source 1..21: mol_type = other DNA
ccgccagattctactcagaaa

SEQ ID NO: 86 - DNA, 21 bp, synthetic construct
  misc_feature 1..21: note = synthetic sequence
  source 1..21: mol_type = other DNA
tgggatgtaattgatattatt

SEQ ID NO: 87 - DNA, 21 bp, synthetic construct
  misc_feature 1..21: note = synthetic sequence
  source 1..21: mol_type = other DNA
aaggctagttatgatagttaa

SEQ ID NO: 88 - DNA, 21 bp, synthetic construct
  misc_feature 1..21: note = synthetic sequence
  source 1..21: mol_type = other DNA
ctggagaacattgcaacatta

SEQ ID NO: 89 - DNA, 21 bp, synthetic construct
  misc_feature 1..21: note = synthetic sequence
  source 1..21: mol_type = other DNA
tccgggaaatatgggaactaa

SEQ ID NO: 90 - DNA, 21 bp, synthetic construct
  misc_feature 1..21: note = synthetic sequence
  source 1..21: mol_type = other DNA
ctggatagaatgattgctgaa

SEQ ID NO: 91 - DNA, 21 bp, synthetic construct
  misc_feature 1..21: note = synthetic sequence
  source 1..21: mol_type = other DNA
cacgggaacttgatcctagaa

SEQ ID NO: 92 - DNA, 21 bp, synthetic construct
  misc_feature 1..21: note = synthetic sequence
  source 1..21: mol_type = other DNA
caaggcaaatccaatacggaa

SEQ ID NO: 93 - DNA, 21 bp, synthetic construct
  misc_feature 1..21: note = synthetic sequence
  source 1..21: mol_type = other DNA
cagaggatgcactatcattaa

SEQ ID NO: 94 - DNA, 21 bp, synthetic construct
  misc_feature 1..21: note = synthetic sequence
  source 1..21: mol_type = other DNA
caggttgaagccttccacaaa